European Patent Specification EP 3 455 379 B1, published July 5, 2023. Title: Ribonucleic acid (RNA) interactions. Applicant: Agency for Science, Technology and Research. The sequence listing filed with the application follows.

SEQUENCE LISTING (74 sequences)

SEQ ID NO: 1 - DNA, 17 bp, Artificial Sequence
  custom sequence
ctgtaggcaccatcaat

SEQ ID NO: 2 - DNA, 96 bp, Artificial Sequence
  custom sequence
  iSp18 (49)..(50): iSp18 position
  iSp18 (55)..(56): iSp18 position
agatcggaagagcgtcgtgtagggaaagagtgtagatctcggtggtcgccactcattcagacgtgtgctcttccgatctattgatggtgcctacag

SEQ ID NO: 3 - DNA, 20 bp, Artificial Sequence
  custom sequence
ctggcaggatcaaccaggta

SEQ ID NO: 4 - DNA, 20 bp, Artificial Sequence
  custom sequence
gggcggtggctcgcctcgcg

SEQ ID NO: 5 - DNA, 20 bp, Artificial Sequence
  custom sequence
tgacccgcacttactgggaa

SEQ ID NO: 6 - DNA, 21 bp, Artificial Sequence
  custom sequence
aatgatccttccgcaggttca

SEQ ID NO: 7 - DNA, 20 bp, Artificial Sequence
  custom sequence
acgtctgatctgaggtcgcg

SEQ ID NO: 8 - DNA, 22 bp, Artificial Sequence
  custom sequence
tggtccgtgtttcaagacgggt

SEQ ID NO: 9 - DNA, 22 bp, Artificial Sequence
  custom sequence
caagacctctaatcattcgctt

SEQ ID NO: 10 - DNA, 21 bp, Artificial Sequence
  custom sequence
tgtcgagggctgactttcaat

SEQ ID NO: 11 - DNA, 21 bp, Artificial Sequence
  custom sequence
tgcttagcttccgagatcaga

SEQ ID NO: 12 - DNA, 21 bp, Artificial Sequence
  custom sequence
aagcctacagcacccggtatt

SEQ ID NO: 13 - DNA, 23 bp, Artificial Sequence
  custom sequence
gtaagaacacagcctgtggtaag

SEQ ID NO: 14 - DNA, 20 bp, Artificial Sequence
  custom sequence
tcctctttctatacagtcag

SEQ ID NO: 15 - DNA, 20 bp, Artificial Sequence
  custom sequence
atatggggtaggtttactct

SEQ ID NO: 16 - DNA, 20 bp, Artificial Sequence
  custom sequence
gaggaaaagcgaagcgaggc

SEQ ID NO: 17 - DNA, 20 bp, Artificial Sequence
  custom sequence
gcgaatgcttgtggaatgta

SEQ ID NO: 18 - DNA, 20 bp, Artificial Sequence
  custom sequence
aacttgatccaacctctttg

SEQ ID NO: 19 - DNA, 20 bp, Artificial Sequence
  custom sequence
ggcaaacccgttgcgaaaaa

SEQ ID NO: 20 - DNA, 20 bp, Artificial Sequence
  custom sequence
tagttttcacgacacctgtg

SEQ ID NO: 21 - DNA, 20 bp, Artificial Sequence
  custom sequence
accactgattaagagtgggg

SEQ ID NO: 22 - DNA, 20 bp, Artificial Sequence
  custom sequence
acatgatctgggtcatcttc

SEQ ID NO: 23 - DNA, 20 bp, Artificial Sequence
  custom sequence
ggatagcacagcctggatag

SEQ ID NO: 24 - DNA, 20 bp, Artificial Sequence
  custom sequence
atctcttgctcgaagtccag

SEQ ID NO: 25 - DNA, 20 bp, Artificial Sequence
  custom sequence
tcattgccaatggtgatgac

SEQ ID NO: 26 - DNA, 20 bp, Artificial Sequence
  custom sequence
ctcaggaggagcaatgatct

SEQ ID NO: 27 - DNA, 20 bp, Artificial Sequence
  custom sequence
cacattgtgaactttggggg

SEQ ID NO: 28 - DNA, 20 bp, Artificial Sequence
  custom sequence
gacttcctgtaacaacgcat

SEQ ID NO: 29 - DNA, 20 bp, Artificial Sequence
  custom sequence
gtctcaagtcagtgtacagg

SEQ ID NO: 30 - DNA, 20 bp, Artificial Sequence
  custom sequence
acccatgtttagttaattat

SEQ ID NO: 31 - DNA, 20 bp, Artificial Sequence
  custom sequence
tcgacatgaccgataacgac

SEQ ID NO: 32 - DNA, 20 bp, Artificial Sequence
  custom sequence
accaccacacttgtaaatca

SEQ ID NO: 33 - DNA, 20 bp, Artificial Sequence
  custom sequence
cacggattatttgcctgatt

SEQ ID NO: 34 - DNA, 20 bp, Artificial Sequence
  custom sequence
attttgcgtaacctattcgc

SEQ ID NO: 35 - DNA, 20 bp, Artificial Sequence
  custom sequence
ttagagggacaagtggcgtt

SEQ ID NO: 36 - DNA, 20 bp, Artificial Sequence
  custom sequence
ggacatctaagggcatcaca

SEQ ID NO: 37 - DNA, 20 bp, Artificial Sequence
  custom sequence
gagaactttgaaggccgaag

SEQ ID NO: 38 - DNA, 20 bp, Artificial Sequence
  custom sequence
catctctcaggaccgactga

SEQ ID NO: 39 - DNA, 22 bp, Artificial Sequence
  custom sequence
gcgcccgatctcgtctgatctc

SEQ ID NO: 40 - DNA, 21 bp, Artificial Sequence
  custom sequence
caggcggtctcccatccaagt

SEQ ID NO: 41 - DNA, 22 bp, Artificial Sequence
  custom sequence
caggctgtgttcttacactgac

SEQ ID NO: 42 - DNA, 22 bp, Artificial Sequence
  custom sequence
atgttcccccattcacaataca

SEQ ID NO: 43 - DNA, 21 bp, Artificial Sequence
  custom sequence
ggtcattaccaaggcttttag

SEQ ID NO: 44 - DNA, 21 bp, Artificial Sequence
  custom sequence
gcagatagaaaacctactggg

SEQ ID NO: 45 - DNA, 22 bp, Artificial Sequence
  custom sequence
tcagagtgagcgctgggtacag

SEQ ID NO: 46 - DNA, 20 bp, Artificial Sequence
  custom sequence
ggaaggcagtagagaatggt

SEQ ID NO: 47 - DNA, 20 bp, Artificial Sequence
  custom sequence
cgatatggctgagatcgaga

SEQ ID NO: 48 - DNA, 20 bp, Artificial Sequence
  custom sequence
ctttggaaggcagtggattt

SEQ ID NO: 49 - DNA, 20 bp, Artificial Sequence
  custom sequence
ctgtcaaggatgttcgtcgt

SEQ ID NO: 50 - DNA, 20 bp, Artificial Sequence
  custom sequence
cttatttggcctggatggtt

SEQ ID NO: 51 - DNA, 20 bp, Artificial Sequence
  custom sequence
tcgcaaaggatctccttcat

SEQ ID NO: 52 - DNA, 19 bp, Artificial Sequence
  custom sequence
ccaggcgtttcttcttgtg

SEQ ID NO: 53 - DNA, 20 bp, Artificial Sequence
  custom sequence
actctgcattctcgcttcct

SEQ ID NO: 54 - DNA, 20 bp, Artificial Sequence
  custom sequence
ctcgtttgtacccgttgatg

SEQ ID NO: 55 - DNA, 20 bp, Artificial Sequence
  custom sequence
tggtatcgtggaaggactca

SEQ ID NO: 56 - DNA, 20 bp, Artificial Sequence
  custom sequence
ccagtagaggcagggatgat

SEQ ID NO: 57 - DNA, 19 bp, Artificial Sequence
  custom sequence
agagaggcatcctcaccct

SEQ ID NO: 58 - DNA, 20 bp, Artificial Sequence
  custom sequence
cacacgcagctcattgtaga

SEQ ID NO: 59 - DNA, 20 bp, Artificial Sequence
  custom sequence
gaaggaggagctgctgaaac

SEQ ID NO: 60 - DNA, 21 bp, Artificial Sequence
  custom sequence
tcggatcttagagagcttgga

SEQ ID NO: 61 - DNA, 20 bp, Artificial Sequence
  custom sequence
gactttgtcacagcccaaga

SEQ ID NO: 62 - DNA, 20 bp, Artificial Sequence
  custom sequence
caagcaagcagaatttggaa

SEQ ID NO: 63 - DNA, 20 bp, Artificial Sequence
  custom sequence
gaatcagaaagcggtggatt

SEQ ID NO: 64 - DNA, 19 bp, Artificial Sequence
  custom sequence
accagaccagggatgagtg

SEQ ID NO: 65 - DNA, 23 bp, Artificial Sequence
  custom sequence
catgggtaaagagaagtctcaca

SEQ ID NO: 66 - DNA, 22 bp, Artificial Sequence
  custom sequence
ggttctcttgtcaataccacca

SEQ ID NO: 67 - DNA, 21 bp, Artificial Sequence
  custom sequence
gattcgctgtcagagacatga

SEQ ID NO: 68 - DNA, 20 bp, Artificial Sequence
  custom sequence
cagccttggtaaccttagcg

SEQ ID NO: 69 - DNA, 20 bp, Artificial Sequence
  custom sequence
gagaaggatgtggtccgagt

SEQ ID NO: 70 - DNA, 20 bp, Artificial Sequence
  custom sequence
gtgcatagtcgctgcttgat

SEQ ID NO: 71 - DNA, 20 bp, Artificial Sequence
  custom sequence
gctggtagggagtcagaagg

SEQ ID NO: 72 - DNA, 20 bp, Artificial Sequence
  custom sequence
ttggtttccttcctggagtt

SEQ ID NO: 73 - DNA, 20 bp, Artificial Sequence
  custom sequence
tcaagaaggtggtgaagcag

SEQ ID NO: 74 - DNA, 20 bp, Artificial Sequence
  custom sequence
cgctgttgaagtcagaggag